European Patent Application EP 4 692 373 A1, published February 11, 2026. Title: Use of methylation level detection of TXNRD1 gene in diagnosis and/or screening of endometrial cancer. Applicant: BEIJING USCI MEDICAL LABORATORY CO., LTD. The sequence listing filed with the application follows.

SEQUENCE LISTING (21 sequences)

SEQ ID NO: 1 - DNA, 25 bp, synthetic construct
  source 1..25: mol_type = other DNA
ttttttttaataggaaagaacggtc

SEQ ID NO: 2 - DNA, 19 bp, synthetic construct
  source 1..19: mol_type = other DNA
gatcaatcctcccacctcg

SEQ ID NO: 3 - DNA, 16 bp, synthetic construct
  source 1..16: mol_type = other DNA
tcggttgggcgcggtg

SEQ ID NO: 4 - DNA, 18 bp, synthetic construct
  source 1..18: mol_type = other DNA
acgtttggcggaggtcgc

SEQ ID NO: 5 - DNA, 21 bp, synthetic construct
  source 1..21: mol_type = other DNA
cttcgctattatcaccgaacg

SEQ ID NO: 6 - DNA, 15 bp, synthetic construct
  source 1..15: mol_type = other DNA
ttgtcggtcgcgggt

SEQ ID NO: 7 - DNA, 18 bp, synthetic construct
  source 1..18: mol_type = other DNA
agtttcgttggggcggtc

SEQ ID NO: 8 - DNA, 19 bp, synthetic construct
  source 1..19: mol_type = other DNA
caaacgtccttcgactccg

SEQ ID NO: 9 - DNA, 20 bp, synthetic construct
  source 1..20: mol_type = other DNA
ttcggcgtagtttatgtcgt

SEQ ID NO: 10 - DNA, 19 bp, synthetic construct
  source 1..19: mol_type = other DNA
cggtcggaaggttcgtttc

SEQ ID NO: 11 - DNA, 19 bp, synthetic construct
  source 1..19: mol_type = other DNA
aaaacgacgataaccgccg

SEQ ID NO: 12 - DNA, 20 bp, synthetic construct
  source 1..20: mol_type = other DNA
ttttcgttttcggtcgtatt

SEQ ID NO: 13 - DNA, 21 bp, synthetic construct
  source 1..21: mol_type = other DNA
cgagatttcggttcggttttc

SEQ ID NO: 14 - DNA, 19 bp, synthetic construct
  source 1..19: mol_type = other DNA
cgaaaaacgaaaaccgacg

SEQ ID NO: 15 - DNA, 16 bp, synthetic construct
  source 1..16: mol_type = other DNA
ctaccccgcccgctaa

SEQ ID NO: 16 - DNA, 22 bp, synthetic construct
  source 1..22: mol_type = other DNA
ggtattttcggattcggttgtc

SEQ ID NO: 17 - DNA, 19 bp, synthetic construct
  source 1..19: mol_type = other DNA
aacgacccgcctaatttcg

SEQ ID NO: 18 - DNA, 17 bp, synthetic construct
  source 1..17: mol_type = other DNA
acccgttaaaacgtcct

SEQ ID NO: 19 - DNA, 25 bp, synthetic construct
  source 1..25: mol_type = other DNA
gggaagatgggatagaagggaatat

SEQ ID NO: 20 - DNA, 22 bp, synthetic construct
  source 1..22: mol_type = other DNA
aacaattataaactccaaccac

SEQ ID NO: 21 - DNA, 20 bp, synthetic construct
  source 1..20: mol_type = other DNA
ttcattctaacccaatacct